European Patent Application EP 4 177 272 A1, published May 10, 2023. Title: USE OF REGULATOR OF ITPRIPLI IN PREPARATION OF DRUG THAT REGULATES IMMUNE RESPONSES OR FIGHTS TUMORS. Applicant: FUDAN UNIVERSITY. The sequence listing filed with the application follows.

SEQUENCE LISTING (82 sequences)

SEQ ID NO: 1 - protein, 79 aa, Homo sapiens
HPLMVSDRMDLDTLARSRQLEKRMSEEMRLLEMEFEERKRAAEQRQKAENFWTGDTSSDQLVLGKKDMGWPFQADGQEG

SEQ ID NO: 2 - protein, 54 aa, Homo sapiens
DRMDLDTLARSRQLEKRMSEEMRLLEMEFEERKRAAEQRQKAENFWTGDTSSDQ

SEQ ID NO: 3 - protein, 42 aa, Homo sapiens
MDLDTLARSRQLEKRMSEEMRLLEMEFEERKRAAEQRQKAEN

SEQ ID NO: 4 - protein, 103 aa, Homo sapiens
MNVDAEASMAVISLLFLAVMYVVHHPLMVSDRMDLDTLARSRQLEKRMSEEMRLLEMEFEERKRAAEQRQKAENFWTGDTSSDQLVLGKKDMGWPFQADGQEG

SEQ ID NO: 5 - protein, 310 aa, Homo sapiens
HPLMVSDRMDLDTLARSRQLEKRMSEEMRLLEMEFEERKRAAEQRQKAENFWTGDTSSDQLVLGKKDMGWPFQADGQEGPKSCDKTHTCPPCPAPELLGGPSVFLFPPKPKDTLMISRTPEVTCVVVDVSHEDPEVKFNWYVDGVEVHNAKTKPREEQYNSTYRVVSVLTVLHQDWLNGKEYKCKVSNKALPAPIEKTISKAKGQPREPQVYTLPPSRDELTKNQVSLTCLVKGFYPSDIAVEWESNGQPENNYKTTPPVLDSDGSFFLYSKLTVDKSRWQQGNVFSCSVMHEALHNHYTQKSLSLSPGK

SEQ ID NO: 6 - protein, 285 aa, Homo sapiens
DRMDLDTLARSRQLEKRMSEEMRLLEMEFEERKRAAEQRQKAENFWTGDTSSDQPKSCDKTHTCPPCPAPELLGGPSVFLFPPKPKDTLMISRTPEVTCVVVDVSHEDPEVKFNWYVDGVEVHNAKTKPREEQYNSTYRVVSVLTVLHQDWLNGKEYKCKVSNKALPAPIEKTISKAKGQPREPQVYTLPPSRDELTKNQVSLTCLVKGFYPSDIAVEWESNGQPENNYKTTPPVLDSDGSFFLYSKLTVDKSRWQQGNVFSCSVMHEALHNHYTQKSLSLSPGK

SEQ ID NO: 7 - protein, 273 aa, Homo sapiens
MDLDTLARSRQLEKRMSEEMRLLEMEFEERKRAAEQRQKAENPKSCDKTHTCPPCPAPELLGGPSVFLFPPKPKDTLMISRTPEVTCVVVDVSHEDPEVKFNWYVDGVEVHNAKTKPREEQYNSTYRVVSVLTVLHQDWLNGKEYKCKVSNKALPAPIEKTISKAKGQPREPQVYTLPPSRDELTKNQVSLTCLVKGFYPSDIAVEWESNGQPENNYKTTPPVLDSDGSFFLYSKLTVDKSRWQQGNVFSCSVMHEALHNHYTQKSLSLSPGK

SEQ ID NO: 8 - DNA, 1710 bp, Homo sapiens
gaattcgccaccatgaatgttgatgcagaggcctccatggctgtgataagcctgctgttcttggcagtgatgtatgttgttcaccaccctctgatggtcagtgatcggatggacctggacacattagccaggagtcggcagctggagaagcgaatgagtgaggagatgcgcctgctagagatggagtttgaagagagaaagcgagccgctgagcagaggcagaaggcagagaacttctggacaggagacacatccagtgaccagttagtgctggggaagaaagacatggggtggccgttccaggccgatggccaggaagggcctctgggctggatgctgggaaacctgtggaacactggcctcttttgcctttttctcgtctttgagctcctgcgacagaacatgcagcatgaaccggcctttgattccagcagtgaggaggaggaggaggaagtccgtgttgtccctgtcacctcttacaactggcttactgacttcccctcccaggaggccctggactccttttacaaacactatgtccaaaatgccatccgtgacctgccctgcacctgtgagtttgtggagagttttgtggatgatctcattgaggcctgtcgggtgctcagccgccaagaggctcacccacaattggaagactgcctgggcatcggggctgcctttgagaaatggggaaccctccatgagacccagaaatttgatatcctggtgcccattgtccccccacagggcaccatgtttgtcctggagatgagggacccagccctgggccgccgctgtggctgtgtgctggtggagtcagaatgtgtgtgcaagcgtgagaaactcctaggggacgtgctgtgcctggtgcaccaccacagggacccctcggcagtcttggggaagtgtagtagctccatcaaggcagctctctgcaccggcttccacctagacgtgtgcaagactgtgcagtggttccggaacatgatgggcaatgcctgggcccttgtggcccacaagtatgactttaaactcagtctcccaccgtctaccacctcctgcaagctccggctggactatcgctcaggccgctttctctcaatccacttggtcctgggggtgcaacgagaagacaccttggtctacctggtgagtcaggctcctgaccaggagcagctcaccagtgtggactggcctgagtcctttgtggcctgtgagcacctgttcctgaagctggtggggcgctttgcccccgagaacacctgtcacctcaagtgcctccagatcattttaagtctccggcagcatcagagcttaccccatggagcatcccgccccatcctcacttcttaccattttaaaacagctctcatgcacctcttgctacggctgcccctcacggactgggcccacaacatgctctctcagcggctccaggacattctctggttcttgggccgtggcctccagcaaaggtccctccatcatttcctcattggtaacaattttctgcccctgaccatcccaatccctaagacatttaggaatgctgagccggtcaatctcttccaacacctggtgctcaaccccaaggcacattcacaggcagtggaagagttccaaaaccttctgacccaggtgaaaactctgcctcatgccccactggctgcagcacctgattacaaggatgacgacgataagtgactcgag

SEQ ID NO: 9 - DNA, 237 bp, Homo sapiens
cacccactgatggtgagcgaccgcatggacctcgacacactcgcccggtcacgacagctagaaaagcggatgtctgaggagatgagactgctggagatggagttcgaggagcgcaagcgcgccgccgagcagaggcagaaggccgagaacttctggaccggcgacacatcctctgaccagctcgtgctcggcaagaaggacatgggctggcctttccaggccgacggccaggagggc

SEQ ID NO: 10 - DNA, 162 bp, Homo sapiens
gaccgcatggacctcgacacactcgcccggtcacgacagctagaaaagcggatgtctgaggagatgagactgctggagatggagttcgaggagcgcaagcgcgccgccgagcagaggcagaaggccgagaacttctggaccggcgacacatcctctgaccag

SEQ ID NO: 11 - DNA, 20 bp, Artificial Sequence
  synthetic oligonucleotide
ccccagcactaactggtcac

SEQ ID NO: 12 - DNA, 20 bp, Artificial Sequence
  synthetic oligonucleotide
agacatggggtggccgttcc

SEQ ID NO: 13 - DNA, 20 bp, Artificial Sequence
  synthetic oligonucleotide
tcctggccatcggcctggaa

SEQ ID NO: 14 - DNA, 25 bp, Artificial Sequence
  synthetic oligonucleotide
caccgccccagcactaactggtcac

SEQ ID NO: 15 - DNA, 25 bp, Artificial Sequence
  synthetic oligonucleotide
aaacgtgaccagttagtgctggggc

SEQ ID NO: 16 - DNA, 25 bp, Artificial Sequence
  synthetic oligonucleotide
caccgagacatggggtggccgttcc

SEQ ID NO: 17 - DNA, 25 bp, Artificial Sequence
  synthetic oligonucleotide
aaacggaacggccaccccatgtctc

SEQ ID NO: 18 - DNA, 25 bp, Artificial Sequence
  synthetic oligonucleotide
caccgtcctggccatcggcctggaa

SEQ ID NO: 19 - DNA, 25 bp, Artificial Sequence
  synthetic oligonucleotide
aaacttccaggccgatggccaggac

SEQ ID NO: 20 - protein, 538 aa, Artificial Sequence
  synthetic peptide
HPLMVSDRMDLDTLARSRQLEKRMSEEMRLLEMEFEERKRAAEQRQKAENFWTGDTSSDQLVLGKKDMGWPFQADGQEGPLGWMLGNLWNTGLFCLFLVFELLRQNMQHEPAFDSSSEEEEEEVRVVPVTSYNWLTDFPSQEALDSFYKHYVQNAIRDLPCTCEFVESFVDDLIEACRVLSRQEAHPQLEDCLGIGAAFEKWGTLHETQKFDILVPIVPPQGTMFVLEMRDPALGRRCGCVLVESECVCKREKLLGDVLCLVHHHRDPSAVLGKCSSSIKAALCTGFHLDVCKTVQWFRNMMGNAWALVAHKYDFKLSLPPSTTSCKLRLDYRSGRFLSIHLVLGVQREDTLVYLVSQAPDQEQLTSVDWPESFVACEHLFLKLVGRFAPENTCHLKCLQIILSLRQHQSLPHGASRPILTSYHFKTALMHLLLRLPLTDWAHNMLSQRLQDILWFLGRGLQQRSLHHFLIGNNFLPLTIPIPKTFRNAEPVNLFQHLVLNPKAHSQAVEEFQNLLTQVKTLPHAPLAAAPDYKDDDK

SEQ ID NO: 21 - protein, 310 aa, Artificial Sequence; identical to SEQ ID NO: 5
  synthetic peptide

SEQ ID NO: 22 - protein, 461 aa, Artificial Sequence
  synthetic peptide
MEWRIFLFILSGTAGVHSQVQLQQSGPELVKPGASVRMSCKTSGYTFTDYVISWVKQRPGQGLEWIGEIFPRTGSTYYNENFKATATLTADKSSNTAYMQLSSLTSEDSAAYFCAFITSVDWAMEYWGQGTSVTVSSAKTTPPSVYPLAPGSAAQTNSMVTLGCLVKGYFPEPVTVTWNSGSLSSGVHTFPAVLQSDLYTLSSSVTVPSSTWPSETVTCNVAHPASSTKVDKKIVPRDCGCKPCICTVPEVSSVFIFPPKPKDVLTITLTPKVTCVVVDISKDDPEVQFSWFVDDVEVHTAQTQPREEQFNSTFRSVSELPIMHQDWLNGKEFKCRVNSAAFPAPIEKTISKTKGRPKAPQVYTIPPPKEQMAKDKVSLTCMITDFFPEDITVEWQWNGQPAENYKNTQPIMDTDGSYFVYSKLNVQKSNWEAGNTFTCSVLHEGLHNHHTEKSLSHSPGK

SEQ ID NO: 23 - protein, 238 aa, Artificial Sequence
  synthetic peptide
MKLPVRLLVLMFWIPGSSSDVVMTQTPLSLPVSLGDQASISCRSSESLVNSKGNTHLHWYLQKPGQSPKLLIYKVSNRFSGVPDRFSGSGSGTDFTLKISRVEAEDLGVYFCSQSTHAPYTFGGGTKLEIKRADAAPTVSIFPPSSEQLTSGGASVVCFLNNFYPKDINVKWKIDGSERQNGVLNSWTDQDSKDSTYSMSSTLTLTKDEYERHNSYTCEATHKTSTSPIVKSFNRNEC

SEQ ID NO: 24 - protein, 119 aa, Artificial Sequence
  synthetic peptide
QVQLQQSGPELVKPGASVRMSCKTSGYTFTDYVISWVKQRPGQGLEWIGEIFPRTGSTYYNENFKATATLTADKSSNTAYMQLSSLTSEDSAAYFCAFITSVDWAMEYWGQGTSVTVSS

SEQ ID NO: 25 - protein, 113 aa, Artificial Sequence
  synthetic peptide
DVVMTQTPLSLPVSLGDQASISCRSSESLVNSKGNTHLHWYLQKPGQSPKLLIYKVSNRFSGVPDRFSGSGSGTDFTLKISRVEAEDLGVYFCSQSTHAPYTFGGGTKLEIKR

SEQ ID NO: 26 - protein, 8 aa, Artificial Sequence
  synthetic peptide
GYTFTDYV

SEQ ID NO: 27 - protein, 8 aa, Artificial Sequence
  synthetic peptide
IFPRTGST

SEQ ID NO: 28 - protein, 12 aa, Artificial Sequence
  synthetic peptide
AFITSVDWAMEY

SEQ ID NO: 29 - protein, 11 aa, Artificial Sequence
  synthetic peptide
ESLVNSKGNTH

SEQ ID NO: 30 - protein, 2 aa, Artificial Sequence
  synthetic peptide
KV

SEQ ID NO: 31 - protein, 9 aa, Artificial Sequence
  synthetic peptide
SQSTHAPYT

SEQ ID NO: 32 - protein, 461 aa, Artificial Sequence
  synthetic peptide
MEWRIFLFILSGTAGVHSQVQLQQSGPELVKPGASVKMSCKASGYTFTDYVISWVKQRTGQGLEWIGEIFPRTGSTYFNENFKAKATLTADKSSNTAYMQLSSLTSEDSAAYFCAFITSVDWAMEYWGQGTSVTVSSAKTTPPSVYPLAPGSAAQTNSMVTLGCLVKGYFPEPVTVTWNSGSLSSGVHTFPAVLQSDLYTLSSSVTVPSSTWPSETVTCNVAHPASSTKVDKKIVPRDCGCKPCICTVPEVSSVFIFPPKPKDVLTITLTPKVTCVVVDISKDDPEVQFSWFVDDVEVHTAQTQPREEQFNSTFRSVSELPIMHQDWLNGKEFKCRVNSAAFPAPIEKTISKTKGRPKAPQVYTIPPPKEQMAKDKVSLTCMITDFFPEDITVEWQWNGQPAENYKNTQPIMDTDGSYFVYSKLNVQKSNWEAGNTFTCSVLHEGLHNHHTEKSLSHSPGK

SEQ ID NO: 33 - protein, 238 aa, Artificial Sequence
  synthetic peptide
MKLPVRLLVLMFWIPASSSDVVMTQIPLSLPVSLGDQASISCRSSQSLANSKGNTHLHWYLQKPGQSPKLLIYKVSNRFSGVPDRFSGSGSGTDFTLKISRVEAEDLGLYFCSQSTHVPYTFGGGTKLEIKRADAAPTVSIFPPSSEQLTSGGASVVCFLNNFYPKDINVKWKIDGSERQNGVLNSWTDQDSKDSTYSMSSTLTLTKDEYERHNSYTCEATHKTSTSPIVKSFNRNEC

SEQ ID NO: 34 - protein, 119 aa, Artificial Sequence
  synthetic peptide
QVQLQQSGPELVKPGASVKMSCKASGYTFTDYVISWVKQRTGQGLEWIGEIFPRTGSTYFNENFKAKATLTADKSSNTAYMQLSSLTSEDSAAYFCAFITSVDWAMEYWGQGTSVTVSS

SEQ ID NO: 35 - protein, 114 aa, Artificial Sequence
  synthetic peptide
DVVMTQIPLSLPVSLGDQASISCRSSQSLANSKGNTHLHWYLQKPGQSPKLLIYKVSNRFSGVPDRFSGSGSGTDFTLKISRVEAEDLGLYFCSQSTHVPYTFGGGTKLEIKRA

SEQ ID NO: 36 - protein, 8 aa, Artificial Sequence
  synthetic peptide
GYTFTDYV

SEQ ID NO: 37 - protein, 8 aa, Artificial Sequence
  synthetic peptide
IFPRTGST

SEQ ID NO: 38 - protein, 12 aa, Artificial Sequence
  synthetic peptide
AFITSVDWAMEY

SEQ ID NO: 39 - protein, 11 aa, Artificial Sequence
  synthetic peptide
QSLANSKGNTH

SEQ ID NO: 40 - protein, 2 aa, Artificial Sequence
  synthetic peptide
KV

SEQ ID NO: 41 - protein, 9 aa, Artificial Sequence
  synthetic peptide
SQSTHVPYT

SEQ ID NO: 42 - protein, 15 aa, Artificial Sequence
  synthetic peptide
HPLMVSDRMDLDTLA

SEQ ID NO: 43 - protein, 15 aa, Artificial Sequence
  synthetic peptide
VSDRMDLDTLARSRQ

SEQ ID NO: 44 - protein, 15 aa, Artificial Sequence
  synthetic peptide
MDLDTLARSRQLEKR

SEQ ID NO: 45 - protein, 15 aa, Artificial Sequence
  synthetic peptide
TLARSRQLEKRMSEE

SEQ ID NO: 46 - protein, 15 aa, Artificial Sequence
  synthetic peptide
SRQLEKRMSEEMRLL

SEQ ID NO: 47 - protein, 15 aa, Artificial Sequence
  synthetic peptide
EKRMSEEMRLLEMEF

SEQ ID NO: 48 - protein, 15 aa, Artificial Sequence
  synthetic peptide
SEEMRLLEMEFEERK

SEQ ID NO: 49 - protein, 15 aa, Artificial Sequence
  synthetic peptide
RLLEMEFEERKRAAE

SEQ ID NO: 50 - protein, 15 aa, Artificial Sequence
  synthetic peptide
MEFEERKRAAEQRQK

SEQ ID NO: 51 - protein, 15 aa, Artificial Sequence
  synthetic peptide
ERKRAAEQRQKAENF

SEQ ID NO: 52 - protein, 15 aa, Artificial Sequence
  synthetic peptide
AAEQRQKAENFWTGD

SEQ ID NO: 53 - protein, 15 aa, Artificial Sequence
  synthetic peptide
RQKAENFWTGDTSSD

SEQ ID NO: 54 - protein, 15 aa, Artificial Sequence
  synthetic peptide
ENFWTGDTSSDQLVL

SEQ ID NO: 55 - protein, 15 aa, Artificial Sequence
  synthetic peptide
TGDTSSDQLVLGKKD

SEQ ID NO: 56 - protein, 15 aa, Artificial Sequence
  synthetic peptide
SSDQLVLGKKDMGWP

SEQ ID NO: 57 - protein, 15 aa, Artificial Sequence
  synthetic peptide
LVLGKKDMGWPFQAD

SEQ ID NO: 58 - protein, 15 aa, Artificial Sequence
  synthetic peptide
KKDMGWPFQADGQEG

SEQ ID NO: 59 - protein, 15 aa, Artificial Sequence
  synthetic peptide
ALLEMEFEERKRAAE

SEQ ID NO: 60 - protein, 15 aa, Artificial Sequence
  synthetic peptide
RALEMEFEERKRAAE

SEQ ID NO: 61 - protein, 15 aa, Artificial Sequence
  synthetic peptide
RLAEMEFEERKRAAE

SEQ ID NO: 62 - protein, 15 aa, Artificial Sequence
  synthetic peptide
RLLAMEFEERKRAAE

SEQ ID NO: 63 - protein, 15 aa, Artificial Sequence
  synthetic peptide
RLLEAEFEERKRAAE

SEQ ID NO: 64 - protein, 15 aa, Artificial Sequence
  synthetic peptide
RLLEMAFEERKRAAE

SEQ ID NO: 65 - protein, 15 aa, Artificial Sequence
  synthetic peptide
RLLEMEAEERKRAAE

SEQ ID NO: 66 - protein, 15 aa, Artificial Sequence
  synthetic peptide
RLLEMEFAERKRAAE

SEQ ID NO: 67 - protein, 15 aa, Artificial Sequence
  synthetic peptide
RLLEMEFEARKRAAE

SEQ ID NO: 68 - protein, 15 aa, Artificial Sequence
  synthetic peptide
RLLEMEFEEAKRAAE

SEQ ID NO: 69 - protein, 15 aa, Artificial Sequence
  synthetic peptide
RLLEMEFEERARAAE

SEQ ID NO: 70 - protein, 15 aa, Artificial Sequence
  synthetic peptide
RLLEMEFEERKAAAE

SEQ ID NO: 71 - protein, 15 aa, Artificial Sequence
  synthetic peptide
RLLEMEFEERKRAAA

SEQ ID NO: 72 - protein, 15 aa, Artificial Sequence
  synthetic peptide
RLLEMEFEERKQAAE

SEQ ID NO: 73 - protein, 119 aa, Artificial Sequence
  synthetic peptide
QVQLQESGPGLVKPSETLSLTCTTSGYTFTDYVISWVRQPPGKGLEWIGEIFPRTGSTYYNENFKARATLSADKSKNQASLNLDSVSAADTAIYFCAFITSVDWAMEYWGKGSTVTVSS

SEQ ID NO: 74 - protein, 113 aa, Artificial Sequence
  synthetic peptide
DIQMTQSPSSLSASVGDRVTITCRSSESLVNSKGNTHLHWYQQKPGKAPKLLIYKVSNRFSGVPSRFSGSGSGTDFTFTISSLQPEDIATYFCSQSTHAPYTFGPGTKVDIKR

SEQ ID NO: 75 - protein, 116 aa, Artificial Sequence
  synthetic peptide
QVQLVQSGAEVKKPGASVKVSCKTSGYTFTDYVISWVRQAPGQGLEWIGEIFPRTGSTYYNENFKAKATLTADKSTSTAYMELSSLRSEDTAVYFCAFITSVDWAMEYWGQGTLVT

SEQ ID NO: 76 - protein, 113 aa, Artificial Sequence
  synthetic peptide
DVVMTQTPLSLSVTPGQPASISCRSSESLVNSKGNTHLHWYLQKPGQSPKLLIYKVSNRFSGVPDRFSGSGSGTGFTLKISRVEAEDVGVYFCSQSTHAPYTFGGGTKLEIKR

SEQ ID NO: 77 - protein, 119 aa, Artificial Sequence
  synthetic peptide
EVQLVQSGAEVKKPGESLKISCQTFGYTFTDYVISWVRQMPGQGLEWIGEIFPRTGSTYYNENFKAQATLSADKSSSTAYLQWSSLKASDTAMYFCAFITSVDWAMEYWGQGTMVTVSS

SEQ ID NO: 78 - protein, 113 aa, Artificial Sequence
  synthetic peptide
DVVMTQTPLSLPVTPGEPASISCRSSESLVNSKGNTHLHWYLQKPGQSPKLLIYKVSNRFSGVPDRFSGSGSGTDFTLKISRVEAEDVGVYFCSQSTHAPYTFGQGTKLEIKR

SEQ ID NO: 79 - protein, 119 aa, Artificial Sequence
  synthetic peptide
EVTLKESGPVLVKPTETLTLTCTTSGYTFTDYVISWVRQPPGKALEWIGEIFPRTGSTYYNENFKARATLSADKSKSQAVLTMTNMDPVDTATYFCAFITSVDWAMEYWGQGTLVTVSS

SEQ ID NO: 80 - protein, 113 aa, Artificial Sequence
  synthetic peptide
EVVMTQSPATLSLSPGERATLSCRSSESLVNSKGNTHLHWYQQKPGQAPRLLIYKVSNRFSGIPARFSGSGSGTDFTLTISSLEPEDFAVYFCSQSTHAPYTFGQGTKLEIKR

SEQ ID NO: 81 - protein, 119 aa, Artificial Sequence
  synthetic peptide
EVQLVESGGGLVQPGGSLRLSCATSGYTFTDYVISWVRQAPGKGLEWIGEIFPRTGSTYYNENFKARATLSADKSKNTAYLQMNSLRAEDTAVYFCAFITSVDWAMEYWGQGTLVTVSS

SEQ ID NO: 82 - protein, 113 aa, Artificial Sequence
  synthetic peptide
DVQMTQSPSSLSASVGDRVTITCRSSESLVNSKGNTHLHWYQQKPGKAPKLLIYKVSNRFSGVPSRFSGSGSGTDFTLTISSLQPEDFATYFCSQSTHAPYTFGQGTKVEIKR